European Patent Application EP 4 582 562 A1, published July 9, 2025. Title: Method for evaluating risk of developing gastric cancer in patient after eradication of Helicobacter pylori, polynucleotide and kit. Applicant: The Kitasato Institute. The sequence listing filed with the application follows.

SEQUENCE LISTING (13 sequences)

SEQ ID NO: 1 - DNA, 27 bp, synthetic construct
  source 1..27: mol_type = other DNA
atgaacttctatttactcctagcgagc

SEQ ID NO: 2 - DNA, 21 bp, synthetic construct
  source 1..21: mol_type = other DNA
ttaggtggatttccggtgagg

SEQ ID NO: 3 - DNA, 517 bp, Homo sapiens
  source 1..517: mol_type = other DNA
agttacaccaggcatcctggcccaaagtttcccaaatccaggcggctagaggcccactgcttcccaactaccagctgagggggtccgtcccgagaagggagaagaggccgaagaggaaacatgaacttctatttactcctagcgagcagcattctgtgtgccttgattgtcttctggaaatatcgccgctttcagagaaacactggcgaaatgtcatcaaattcaactgctcttgcactagtgagaccctcttcttctgggttaattaacagcaatacagacaacaatcttgcagtctacgacctctctcgggatattttaaataatttcccacactcaatagccaggcagaagcgaatattggtaaacctcagtatggtggaaaacaagctggttgaactggaacatactctacttagcaagggtttcagaggtgcatcacctcaccggaaatccacctaaaagcgtacaggatgtaatgccagtggtggaaatcattaaagacactttgagtaga

SEQ ID NO: 4 - DNA, 1291 bp, Homo sapiens
  source 1..1291: mol_type = genomic DNA
tctactcaaagtgtctttaatgatttccaccactggcattacatcctgtacgcttttaggtggatttccggtgaggtgatgcacctctgaaacccttgctaagtagagtatgttccagttcaaccagcttgttttccaccatactgaggtttaccaatattcgcttctgcctggctattgagtgtgggaaattatttaaaatatcccgagagaggtcgtagactgcaagattgttgtctgtattgctgttaattaacccagaagaagagggtctcactagtgcaagagcagttgaatttgatgacatttcgccagtgtttctctgtaaagaaagggaattatacatacgtagtttatcgaattaagcaatttccaaactaccgaaaaacaacttgtttaatcttggtcaccaaaataaactgatttcccctaatatgtcgagattaaaaatgtattgaattactacattaattcaaaaatatattcttccaaaaccagactgagaaaaaaaatatatgaaagtagccgttagtgacaaagttccatatcctttccttacatttcctgtaaggaaagcagcccagtaggtaaacatatgaacccttgtctttgactcttatctaaaagcacctcacttgtgactttaacaccagaaaatccacattcacactcgaattatttgtgaatgcccagaaagcaccataaaataaagatggtgagattagcaaacagacacgtgggagaggagaagcaagagaagaaagagagaaggtaagattcttaaagtggagagatggtggtggggaatgggcactgacaactgcactttgatctccaatgagtggaaagctgaccatattacttagggacttggggctttttagaagagaccagaactgtcgaatcactggtcagaatacaggaattgcgggagtaagcggtaaaagtctggggctcctttgagcgaaaaggagagatgaggtgatctccccttacctctcattttactgtattttactctcttacatatacactcccaagtccatatactcatctagcttcatctaattcaaatctcccttacattcaccattacctgaaagcggcgatatttccagaagacaatcaaggcacacagaatgctgctcgctaggagtaaatagaagttcatgtttcctcttcggcctcttctcccttctcgggacggaccccctcagctggtagttgggaagcagtgggcctctagccgcctggatttgggaaactttgggccaggatgcctggtgtaact

SEQ ID NO: 5 - DNA, 17 bp, synthetic construct
  source 1..17: mol_type = other DNA
  misc_feature 1: note = modified with FAM
  misc_feature 17: note = modified with non-fluorescent quencher and MGB in this order
ccgctttcatgaaacca

SEQ ID NO: 6 - DNA, 19 bp, synthetic construct
  source 1..19: mol_type = other DNA
  misc_feature 1: note = modified with FAM
  misc_feature 19: note = modified with non-fluorescent quencher and MGB in this order
gccgcattaagagatacac

SEQ ID NO: 7 - DNA, 18 bp, synthetic construct
  source 1..18: mol_type = other DNA
  misc_feature 1: note = modified with FAM
  misc_feature 18: note = modified with non-fluorescent quencher and MGB in this order
ccgctttcagagccacac

SEQ ID NO: 8 - DNA, 18 bp, synthetic construct
  source 1..18: mol_type = other DNA
  misc_feature 1: note = modified with FAM
  misc_feature 18: note = modified with non-fluorescent quencher and MGB in this order
ccgctttcagagaaacca

SEQ ID NO: 9 - DNA, 22 bp, synthetic construct
  source 1..22: mol_type = other DNA
  misc_feature 1: note = modified with FAM
  misc_feature 22: note = modified with non-fluorescent quencher
atcgccgctttcagagaaacca

SEQ ID NO: 10 - DNA, 22 bp, synthetic construct
  source 1..22: mol_type = other DNA
  misc_feature 1: note = modified with FAM
  misc_feature 22: note = modified with non-fluorescent quencher
atcgccgctttcagagacacac

SEQ ID NO: 11 - DNA, 31 bp, Homo sapiens
  source 1..31: mol_type = genomic DNA
gtatgtataattccctttctttacagagaaa

SEQ ID NO: 12 - DNA, 31 bp, Homo sapiens
  source 1..31: mol_type = genomic DNA
ctacgtatgtataattccctttctttacaga

SEQ ID NO: 13 - DNA, 27 bp, Homo sapiens
  source 1..27: mol_type = genomic DNA
gtatgtataattccctttctttacaga